European Patent Specification EP 3 735 409 B1, published June 21, 2023. Title: Enhancement of Nucleic Acid Polymerization by Aromatic Compounds. Applicant: Stratos Genomics, Inc. Kendall Berg Samantha Vellucci Jessica Vellucci. Application PCT. The sequence listing filed with the application follows.

SEQUENCE LISTING (5 sequences)

SEQ ID NO: 1 - protein, 340 aa, Sulfolobus solfataricus
MIVLFVDFDYFYAQVEEVLNPSLKGKPVVVCVFSGRFEDSGVVATANYEARKFGVYAGIPIVEAKKILPNAVYLPWRDLVYWGVSERIMNLLREYSEKIEIASIDEAYLDISDKVRDYREAYNLGLEIKNKILEKEKITVTVGISKNKVFAAVAGRMAKPNGIKVIDDEEVKRLIRELDIADVQGIPYFTAEKLKKLGINKLVDTLSIEFDKLKGMIGEAKAKYLISLARDEYNEPIRTRVRKSIGRTVTMKRNSRNLEEIKPYLFRAIEESYYKLDKRIPKAIHVVAWKSYWNSQYRWSWFPHGISKETAYSESVQLLQQILKKDKRKIRRIGVRFSKF

SEQ ID NO: 2 - protein, 340 aa, Sulfolobus solfataricus
MIVLFVDFDYFYAQVEEVLNPSLKGKPVVVCVFSGRFEDSGVVATANYEARKFGVYAGIPIVRAKKILPNAVYLPWRDLVYWGVSERIMNLLREYSEKIEIASIDEAYLDISDKVRDYREAYNLGLEIKNKILEKEKITVTVGISKNKVFAAVAGRMAKPNGIKVIDDEEVKRLIRELDIADVQGIPYFTAEKLKKLGINKLVDTLSIEFDKLKGMIGEAKAKYLISLARDEYNEPIRTRVRKSIGRTVTMKRNSRNLEEIKPYLFRAIEESYYKLDKRIPKAIHVVAWKSYWNSQYRWSWFPHGISKETAYSESVQLLQQILKKDKRKIRRIGVRFSKF

SEQ ID NO: 3 - protein, 340 aa, Sulfolobus solfataricus
MIVLFVDFDYFYAQVEEVLNPSLKGKPVVVCVFSGRFEDSGVVATANYEARKFGVYAGIPIVRAKKILPNAVYLPWRDLVYWGVSERIMNLLREYSEKIEIASIDEAYLDISDKVRDYREAYNLGLEIKNKILEKEKITVTVGISKNKVFAAVAGRMAKPNGIKVIDDEEVKRLIRELDIADVQGIPYFTAEKLKKLGINKLVDTLSIEFDKLKGMIGEAKAKYLISLARDEYNEPIRTRVRRSIGRTVTMKRNSRNLEEIKPYLFRAIEESYYKLDKRIPKAIHVVAWKSYWNSQYRWSWFPHGISKETAYSESVQLLQQILKKDKRKIRRIGVRFSKF

SEQ ID NO: 4 - protein, 340 aa, Sulfolobus solfataricus
MIVLFVDFDYFYAQVEEVLNPSLKGKPVVVCVFSGRFEDSGVVATANYEARKFGVYAGIPIVRAKKILPNAVYLPWRDLVYWGVSERIMNLLREYSEKIEIASIDEAYLDISDKVRDYREAYNLGLEIKNKILEKEKITVTVGISKNKVFAAVAGRMAKPNGIKVIDDEEVKRLIRELDIADVQGIPYFTAEKLKKLGINKLVDTLSIEFDKLKGMIGEAKAKYLISLARDEYNEPIRTRVRKSIGRTVTMKRDSRNLEEIKPYLFRAIEESYYKLDKRIPKAIHVVAWKSYWNSQYRWSWFPHGISKETAYSESVQLLQQILKKDKRKIRRIGVRFSKF

SEQ ID NO: 5 - protein, 340 aa, Sulfolobus solfataricus
MIVLFVDFDYFYAQVEEVLNPSLKGKPVVVCVFSGRFEDSGVVATANYEARKFGVYAGIPIKRAKKILPNAVYLPWRDLVYWGVSERIMNLLREYSEKIEIASIDEAYLDISDKVRDYREAYNLGLEIKNKILEKEKITVTVGISKNKVFAAVAGRMAKPNGIKVIDDEEVKRLIRELDIADVQGIPYFTAEKLKKLGINKLVDTLSIEFDKLKGMIGEAKAKYLISLARDEYNEPIRTRVRKSIGRTVTMKRNSRNLEEIKPYLFRAIEESYYKLDKRIPKAIHVVAWKSYWNSQYRWSWFPHGISKETAYSESVQLLQQILKKDKRKIRRIGVRFSKF